European Patent Application EP 4 397 678 A2, published July 10, 2024. Title: METHODS AND COMPOSITIONS FOR TREATING LIVER DISEASE. Applicant: UNITED STATES GOVERNMENT AS REPRESENTED BY THE DEPARTMENT OF VETERANS AFFAIRS. The sequence listing filed with the application follows.

SEQUENCE LISTING (15 sequences)

SEQ ID NO: 1 - protein, 121 aa, Homo sapiens
MAPRPLLLLLLLLGGSAARPAPPRARRHSDGTFTSELSRLREGARLQRLLQGLVGKRSEQDAENSMAWTRLSAGLLCPSGSNMPILQAWMPLDGTWSPWLPPGPMVSEPAGAAAEGTLRPR

SEQ ID NO: 2 - protein, 27 aa, Homo sapiens
HSDGTFTSELSRLREGARLQRLLQGLV

SEQ ID NO: 3 - protein, 23 aa, Homo sapiens
TFTSELSRLRKGARLQRLLQGLV

SEQ ID NO: 4 - DNA, 18 bp, synthetic construct
  misc_feature 1..18: note = primer
  source 1..18: mol_type = other DNA
gagtgccaccttgccctg

SEQ ID NO: 5 - DNA, 20 bp, synthetic construct
  misc_feature 1..20: note = primer
  source 1..20: mol_type = other DNA
gatttgagtttcggtgctgg

SEQ ID NO: 6 - DNA, 20 bp, synthetic construct
  misc_feature 1..20: note = primer
  source 1..20: mol_type = other DNA
ggtttggggagccagtatct

SEQ ID NO: 7 - DNA, 20 bp, synthetic construct
  misc_feature 1..20: note = primer
  source 1..20: mol_type = other DNA
caagcctgcattcatcaaga

SEQ ID NO: 8 - DNA, 20 bp, synthetic construct
  misc_feature 1..20: note = primer
  source 1..20: mol_type = other DNA
gccagaggccacttgtgtag

SEQ ID NO: 9 - DNA, 20 bp, synthetic construct
  misc_feature 1..20: note = primer
  source 1..20: mol_type = other DNA
tcatactcaggcccagttcc

SEQ ID NO: 10 - DNA, 17 bp, synthetic construct
  misc_feature 1..17: note = primer
  source 1..17: mol_type = other DNA
cccatggctcaggcaag

SEQ ID NO: 11 - DNA, 22 bp, synthetic construct
  misc_feature 1..22: note = primer
  source 1..22: mol_type = other DNA
gtgcctgaggtttcatactcag

SEQ ID NO: 12 - DNA, 20 bp, synthetic construct
  misc_feature 1..20: note = primer
  source 1..20: mol_type = other DNA
caacacgcgctggaagttca

SEQ ID NO: 13 - DNA, 22 bp, synthetic construct
  misc_feature 1..22: note = primer
  source 1..22: mol_type = other DNA
gatgctgcctagttcaaagtcg

SEQ ID NO: 14 - DNA, 20 bp, synthetic construct
  misc_feature 1..20: note = primer
  source 1..20: mol_type = other DNA
tgtcaagaccgacctgtccg

SEQ ID NO: 15 - DNA, 20 bp, synthetic construct
  misc_feature 1..20: note = primer
  source 1..20: mol_type = other DNA
tattcggcaagcaggcatcg